European Patent Application EP 4 289 431 A1, published December 13, 2023. Title: Composition for preventing or treating of neuroinflammatory disease comprising didanosine. Applicant: OATC Inc Daegu Gyeongbuk Institute of Science and Technology. The sequence listing filed with the application follows.

SEQUENCE LISTING (4 sequences)

SEQ ID NO: 1 - DNA, 1347 bp, Artificial Sequence
  Psen2 N141I
atgctcgcattcatggcctctgacagcgaggaagaggtgtgtgatgagcggacgtccttgatgtcagccgagagccccacatctcgctcctgccaggaaggcaggccaggcccggaggatggagagagcactgcccagtggaggactcaggagagcgaagaagactgtgaagaggacccggaccgctacgcatgcagtggggctcctgggcgaccgtcgggcctggaggaagagctgaccctcaagtatggggcgaagcatgtgatcatgctattcgtgcctgtcacgctgtgtatgatcgtggtggtggccactatcaagtctgtgcgtttctacactgagaagaacgggcagctcatctacacgcccttcacggaggacacgccctcggtgggccagcggctcctcaactccgtgcttatcaccctcatcatgatcagcgtcatcgtagtcatgaccatcttcctcgtggtactctacaagtatcgatgctacaagttcatccatggctggctgatcatgtcctccctgatgctcctcttcttgttcacctacatctacctcggggaagtgctcaagacctacaatgtggccatggactatcccacactcttcctggctgtctggaacttcggggcagtgggcatggtgtgcatccactggaaggggcctctggtgctgcagcaggcttaccttattgtgatcagcgcactcatggccctggtgttcatcaagtacctgccggagtggtctgcctgggtcatcttgggtgccatctctgtgtacgatctcgtggccgtgctgtgccccaaagggccactgaggatgctggtggaaactgcccaggagagaaatgagcccatatttcctgccctgatatactcatctgccatggtgtggacggtgggcatggcaaagctggacccctcctctcaaggagcgctgcagctcccctatgacccagagatggaagaagactcctacgacagttttggagaaccctcataccctgaagccttcgaagcccccctgcctggctacccaggggaggagctggaggaggaggaggaaaggggcgtgaagctcggcctgggagacttcatcttctacagcgtcctggtgggcaaggctgcagccactggcaacggagactggaacactacgctggcctgttttatcgccatcctcattggcttgtgtctcaccctcctgctgcttgctgtgttcaagaaggctctgcccgccctccccatctccatcacctttggactcatcttctacttctccacagacaacctggtgcgccctttcatggacactctggcctcccaccagctctacatctga

SEQ ID NO: 2 - DNA, 1347 bp, Artificial Sequence; identical to SEQ ID NO: 1
  Psen2 wild type

SEQ ID NO: 3 - DNA, 23 bp, Artificial Sequence
  Primer(F) for IL-6
ctggatataatcaggaaatttgc

SEQ ID NO: 4 - DNA, 22 bp, Artificial Sequence
  Primer(R) for IL-6
aaatcttttacctcttggttga